European Patent Specification EP 4 039 695 B1, published July 30, 2025. Title: EXPRESSION CONSTRUCTS AND METHODS OF GENETICALLY ENGINEERING METHYLOTROPHIC YEAST. Applicant: Impossible Foods Inc. The sequence listing filed with the application follows.

SEQUENCE LISTING (58 sequences)

SEQ ID NO: 1 - DNA, 3486 bp, Komagataella phaffii
atgcgagaccgcggccgcatgagcaatctacccccaacttttggttccactagacaatctccagaagaccaatcacctcccgtgcccaaggagctgtcattcaatgggaccacaccctcaggaaagctacgcttatttgtctgtcagacatgtactcgagcatttgctcgtcaggaacacttgaaacgacacgaaaggtctcacaccaaggagaaacctttcagctgcggcatttgttctcgtaaattcagccgtcgagatctgttattgagacatgcccaaaaactgcacagcaactgctctgatgcggccataacaagactaaggcgcaaggcaactcgtcggtcttctaatgccgcgggttccatatctggttctactccggtgacaacgccaaatactatgggtacgcccgaagatggcgagaaacgaaaagttcagaaactggccggccgccgggactcaaatgaacagaaactgcaactgcaacaacaacatctacagcaacaaccacagttgcaataccaacaatctcttaagcagcatgaaaatcaagtccagcagcctgatcaagatccattgatatccccgagaatgcaattattcaatgattccaaccatcacgtaaacaatttgtttgatcttggactaagaagagcttccttctccgccgttagtggaaataattatgcccattatgtgaataattttcaacaagatgcctcttctaccaatccaaatcaagattcaaataatgccgaatttgagaatattgaattttctaccccacaaatgatgcccgttgaagatgctgaaacttggatgaacaacatgggtccaattccgaacttctctctcgatgtgaacaggaacattggtgatagctttacagatatacaacacaagaattcagagcctattatatccgaaccgcccaaggacaccgctccaaacgacaagaagttgaatggctactctttttacgaagcccccatcaagccattagaatccctattttctgtcaggaatacaaagagaaacaagtataaaacaaatgacgactctccagacaccgtggataataactccgcaccggctgctaataccattcaagaacttgagtcttctttgaatgcatccaagaatttttgcttgccaactggttattccttctatggtaatttggaccaacagactttctctaacacgttatcatgcacttcttctaatgccacaatttcgcccattctactcgataactccattaataataactccactagtgacgtgagaccagaatttagaacacaaagtgtcacctctgaaatgagtcaagcccctccccctcctcaaaaaaacaactcgaaatattccaccgaagttctttttaccagcaacatgcggtcgtttattcactacgctctttccaagtatccttttattggtgtgcccactccaactcttccggagaacgaaagactaaatgaatatgctgattcattcaccaaccgtttcttaaatcattatcctttcatacatgtcacgattctcaaagaatactcccttttcaaggcaattttagatgagaatgagtcgactaagaactgggaaaataatcagttttacttagagaaccaacgaatatcaattgtttgtcttcctcttttggtggctacgataggtgcagtactatcaaacaacaaaaaggatgcttcgaatttatacgaagcttcaaggcgttgtattcatgtttacttagattccaggaaaaagatacccacttccttgtccgcaaataacaatgactctccactttggctaattcaatccctgacgttatctgttatgtatgggttatttgcggacaatgacattagtttgaatgtcgtgatcagacaagttaacgcacttaattctctggtcaagacttcgggcctgaataggacctcaattatagatcttttcaacatcaacaaacctttggataatgaactctggaatcaattcgtgaaaatagagtccaccgtaaggacaatccacacgatttttcaaatcagttccaacttaagcgccttgtacaatattattccatcgttgaaaattgatgacctaatgattactctaccagttcccacaacactttggcaagctgattcttttgtgaaattcaaaagtctaagttacggaaatcagatcccttttcaatatacaagagtactacagaatttgattgattacaatcagccattgagcgatggaaaatttttgtatgaaaaccatgtaagtgagtttggactcatatgcctacagaatggtctacaccaatacagctatttccaaaaattgactgctgtcaataacagagaagatgcgctattcacaaaggttgttaattcacttcacagttgggataggatgatttcgaattctgatttgtttccaaagaagatatatcagcagagttgcttgattttggactcaaagttgcttaataatttcctgattgtcaagagctcattgaaagtttcgaccggagacgttagttctttgaataagttaaaagaaaacgtgtggcttaaaaactggaatcaagtgtgtgctatctattataacagcttcatgaacattcctgctcccagtattcaaaagaagtacaatgacatagagtttgtggatgacatgattaatttgagtctaatcatcatcaagattatgaaactcattttctataacaatgtcaaagacaattatgaggatgaaaatgacttcaaattgcaagagttaaatttaacatttgacaattttgatgagaaaatatccttgaatttgacaatattattcgatatatttttgatgatctacaagataattaccaattacgaaaagtttatgaagatcaaacacaagtttaattactacaattctaattcgaatataagcttcttgcatcatttcgaactctcctcggttatcaataacacccaaatgaaccagaatgattatatgaaaacagatattgatgaaaagcttgatcagcttttccacatctatcaaacatttttccggctgtatctggatttagaaaagtttatgaagttcaaattcaactatcatgactttgagacagagttttcaagtctctcaatatccaatatactgaacactcatgctgcttctaacaatgacacaaatgctgctgatgctatgaatgccaaggatgaaaaaatatctcccacaactttgaatagcgtattacttgctgatgaaggaaatgaaaattccggtcgtaataacgattcagaccgcctgttcatgctgaacgagctaattaattttgaagtaggtttgaaatttctcaagataggtgagtcattttttgatttcttgtatgagaataactacaagttcatccacttcaaaaacttaaatgacggaatgttccacatcaggatatacctagaaaaccgactagatggtggtgtctag

SEQ ID NO: 2 - protein, 1161 aa, Komagataella phaffii
MRDRGRMSNLPPTFGSTRQSPEDQSPPVPKELSFNGTTPSGKLRLFVCQTCTRAFARQEHLKRHERSHTKEKPFSCGICSRKFSRRDLLLRHAQKLHSNCSDAAITRLRRKATRRSSNAAGSISGSTPVTTPNTMGTPEDGEKRKVQKLAGRRDSNEQKLQLQQQHLQQQPQLQYQQSLKQHENQVQQPDQDPLISPRMQLFNDSNHHVNNLFDLGLRRASFSAVSGNNYAHYVNNFQQDASSTNPNQDSNNAEFENIEFSTPQMMPVEDAETWMNNMGPIPNFSLDVNRNIGDSFTDIQHKNSEPIISEPPKDTAPNDKKLNGYSFYEAPIKPLESLFSVRNTKRNKYKTNDDSPDTVDNNSAPAANTIQELESSLNASKNFCLPTGYSFYGNLDQQTFSNTLSCTSSNATISPILLDNSINNNSTSDVRPEFRTQSVTSEMSQAPPPPQKNNSKYSTEVLFTSNMRSFIHYALSKYPFIGVPTPTLPENERLNEYADSFTNRFLNHYPFIHVTILKEYSLFKAILDENESTKNWENNQFYLENQRISIVCLPLLVATIGAVLSNNKKDASNLYEASRRCIHVYLDSRKKIPTSLSANNNDSPLWLIQSLTLSVMYGLFADNDISLNVVIRQVNALNSLVKTSGLNRTSIIDLFNINKPLDNELWNQFVKIESTVRTIHTIFQISSNLSALYNIIPSLKIDDLMITLPVPTTLWQADSFVKFKSLSYGNQIPFQYTRVLQNLIDYNQPLSDGKFLYENHVSEFGLICLQNGLHQYSYFQKLTAVNNREDALFTKVVNSLHSWDRMISNSDLFPKKIYQQSCLILDSKLLNNFLIVKSSLKVSTGDVSSLNKLKENVWLKNWNQVCAIYYNSFMNIPAPSIQKKYNDIEFVDDMINLSLIIIKIMKLIFYNNVKDNYEDENDFKLQELNLTFDNFDEKISLNLTILFDIFLMIYKIITNYEKFMKIKHKFNYYNSNSNISFLHHFELSSVINNTQMNQNDYMKTDIDEKLDQLFHIYQTFFRLYLDLEKFMKFKFNYHDFETEFSSLSISNILNTHAASNNDTNAADAMNAKDEKISPTTLNSVLLADEGNENSGRNNDSDRLFMLNELINFEVGLKFLKIGESFFDFLYENNYKFIHFKNLNDGMFHIRIYLENRLDGGV

SEQ ID NO: 3 - DNA, 438 bp, Artificial Sequence
  Glycine max leghemoglobin codon-optimized for Pichia pastoris
atgggtgctttcaccgagaagcaggaagcacttgtttcctcttcgttcgaagcttttaaggctaacatccctcaatactctgttgtgttttacacgtccattctagaaaaagctcctgctgccaaggacctcttctcttttctgtccaacggtgtagatccatccaatcccaaattaacaggtcacgctgagaaattgttcggtttagtcagagatagcgctggacaattgaaagcaaatggtactgtggttgctgatgctgccttgggcagcatccatgcacagaaggcaattacagacccacaatttgttgttgtgaaggaagctctgcttaaaactataaaggaagccgtcggagacaaatggagtgacgagttgtcatcagcttgggaggtagcttatgatgagttggccgcagcaatcaaaaaggcattctaa

SEQ ID NO: 4 - protein, 145 aa, Artificial Sequence
  Glycine max leghemoglobin codon-optimized for Pichia pastoris
MGAFTEKQEALVSSSFEAFKANIPQYSVVFYTSILEKAPAAKDLFSFLSNGVDPSNPKLTGHAEKLFGLVRDSAGQLKANGTVVADAALGSIHAQKAITDPQFVVVKEALLKTIKEAVGDKWSDELSSAWEVAYDELAAAIKKAF

SEQ ID NO: 5 - DNA, 438 bp, Artificial Sequence
  Glycine max leghemoglobin codon-optimized for Pichia pastoris
atgggtgcatttacagaaaaacaagaggctttagtatcctcatcttttgaagctttcaaagccaatattcctcaatactccgttgttttctatacgtccattttggaaaaggctccagcagctaaggaccttttctctttcttgtcgaacggcgtggatccctcaaatcctaagctgactggtcacgccgagaagctttttggtttggtcagagacagcgccggacagctgaaagctaacggtacagttgtggcagatgctgccttgggatctatacatgcacaaaaggctatcaccgacccacagtttgtggttgtaaaagaggctctactcaaaactatcaaggaagcagttggtgacaaatggagcgatgaattgtccagtgcatgggaggtcgcttacgatgagttagctgctgcaatcaaaaaggctttctaa

SEQ ID NO: 6 - protein, 145 aa, Artificial Sequence; identical to SEQ ID NO: 4
  Glycine max leghemoglobin codon-optimized for Pichia pastoris

SEQ ID NO: 7 - DNA, 939 bp, Pichia pastoris
gatctaacatccaaagacgaaaggttgaatgaaacctttttgccatccgacatccacaggtccattctcacacataagtgccaaacgcaacaggaggggatacactagcagcagaccgttgcaaacgcaggacctccactcctcttctcctcaacacccacttttgccatcgaaaaaccagcccagttattgggcttgattggagctcgctcattccaattccttctattaggctactaacaccatgactttattagcctgtctatcctggcccccctggcgaggttcatgtttgtttatttccgaatgcaacaagctccgcattacacccgaacatcactccagatgagggctttctgagtgtggggtcaaatagtttcatgttccccaaatggcccaaaactgacagtttaaacgctgtcttggaacctaatatgacaaaagcgtgatctcatccaagatgaactaagtttggttcgttgaaatgctaacggccagttggtcaaaaagaaacttccaaaagtcggcataccgtttgtcttgtttggtattgattgacgaatgctcaaaaataatctcattaatgcttagcgcagtctctctatcgcttctgaaccccggtgcacctgtgccgaaacgcaaatggggaaacacccgctttttggatgattatgcattgtctccacattgtatgcttccaagattctggtgggaatactgctgatagcctaacgttcatgatcaaaatttaactgttctaacccctacttgacagcaatatataaacagaaggaagctgccctgtcttaaacctttttttttatcatcattattagcttactttcataattgcgactggttccaattgacaagcttttgattttaacgacttttaacgacaacttgagaagatcaaaaaacaactaattattcgaaacg

SEQ ID NO: 8 - DNA, 558 bp, Pichia pastoris
cgactattatcgatcaatgaaatccatcaagattgaaatcttaaaattgcccctttcacttgacaggatccttttttgtagaaatgtcttggtgtcctcgtccaatcaggtagccatctctgaaatatctggctccgttgcaactccgaacgacctgctggcaacgtaaaattctccggggtaaaacttaaatgtggagtaatggaaccagaaacgtctcttcccttctctctccttccaccgcccgttaccgtccctaggaaattttactctgctggagagcttcttctacggcccccttgcagcaatgctcttcccagcattacgttgcgggtaaaacggaggtcgtgtacccgacctagcagcccagggatggaaaagtcccggccgtcgctggcaataatagcgggcggacgcatgtcatgagattattggaaaccaccagaatcgaatataaaaggcgaacacctttcccaattttggtttctcctgacccaaagactttaaatttaatttatttgtccctatttcaatcaattgaacaactatcaaaacacg

SEQ ID NO: 9 - DNA, 822 bp, Pichia pastoris
caggtgaacccacctaactatttttaactgggatccagtgagctcgctgggtgaaagccaaccatcttttgtttcggggaaccgtgctcgccccgtaaagttaatttttttttcccgcgcagctttaatctttcggcagagaaggcgttttcatcgtagcgtgggaacagaataatcagttcatgtgctatacaggcacatggcagcagtcactattttgctttttaaccttaaagtcgttcatcaatcattaactgaccaatcagattttttgcatttgccacttatctaaaaatacttttgtatctcgcagatacgttcagtggtttccaggacaacacccaaaaaaaggtatcaatgccactaggcagtcggttttatttttggtcacccacgcaaagaagcacccacctcttttaggttttaagttgtgggaacagtaacaccgcctagagcttcaggaaaaaccagtacctgtgaccgcaattcaccatgatgcagaatgttaatttaaacgagtgccaaatcaagatttcaacagacaaatcaatcgatccatagttacccattccagccttttcgtcgtcgagcctgcttcattcctgcctcaggtgcataactttgcatgaaaagtccagattagggcagattttgagtttaaaataggaaatataaacaaatataccgcgaaaaaggtttgtttatagcttttcgcctggtgccgtacggtataaatacatactctcctcccccccctggttctctttttcttttgttacttacattttaccgttccgtcactcgcttcactcaacaacaaaa

SEQ ID NO: 10 - DNA, 424 bp, Pichia pastoris
ataactgtcgcctcttttatctgccgcactgcatgaggtgtccccttagtgggaaagagtactgagccaaccctggaggacagcaagggaaaaatacctacaacttgcttcataatggtcgtaaaaacaatccttgtcggatataagtgttgtagactgtcccttatcctctgcgatgttcttcctctcaaagtttgcgatttctctctatcagaattgccatcaagagactcaggactaatttcgcagtcccacacgcactcgtacatgattggctgaaatttccctaaagaatttctttttcacgaaaattttttttttacacaagattttcagcagatataaaatggagagcaggacctccgctgtgactcttcttttttttcttttattctcactacatacattttagttattcgccaac

SEQ ID NO: 11 - DNA, 1683 bp, Pichia pastoris
atggagtttgtcgcccgtcagtccatgaatgcctgtccctttgtcaggtcaacttctacccaccatttgaagaagttggcagcaaacagttctctagctgctactgctagtcattgtcccgtggttggccctgctctccaacagcagagatactactctcaaccttccaagccagcccaagcccaaacctccgacattgctactgggatcaagaaggatgtttctccgatccgtatggactctaatgaaaccgcctttgattacaatggaatgtatgagtctgatcttgcgaataaacgtaaagataactcgtatcgttatttcaataacatcaaccgtctagccaaggagtttcccaaggcacatcgccagaccgaagatgacaaggtgaccgtctggtgctctaacgactacttaggaatgggtaggcatcctgagattatcaaaaccatgaaggctaccatggacaagtacggttccggagcaggaggaactaggaacattgcaggtcataaccacgccgctatcaatttggaaagcgagttggcttgcttgaacaagaaggaagcggctctggtgttttcatcatgtttcatagctaacgatgcaatcatctcgttgttgggacaaaaaatcaaaaatttggtcattttctctgaccagtcgaatcatgcttccatgatattgggtgtgcgtaactccaaagcgaagaagcacatcttcaagcacaacaatttgaaggatctggagtcgcagttagctcagtaccccaagtcgactcctaaactgatcgccttcgagtcagtttactctatgtgtggatctgtggctcccattgagaagatttgcgatttggctaaaaggtacggtgccctcaccttcttggatgaagttcatgctgttggaatgtatggtcctcatggacagggtgtagctgagcatttggactttgatctgcatttacagtctggaatcgccagtcctagcgtggtggacaaacgcaccatattggatcgtgtcgacatgattactggtacttgcggaaagtcatttggtactgttggaggttacgttgctggtagtgccaacctaattgattggttaagatcctatgcgccaggtttcattttcactaccacacttcctcctgctatcatggctggtacagccacttctgttcgtattgttagggccgacattgaggcccgtatcaagcaacagcttaatactcgctacgtcaaagactcatttgaaaaccttggtattccagtcattccaaacccaagtcacattgttcctgttctagttggaaatgctgcagatgccaagaaggcatccgatatgttaatgaacaaacaccgtatttatgttcaagctattaactaccctactgtgcctgtcggtgaagaacgactaaggattactcctactccaggtcatggaaaggagatttgtgaccagctgatcagcgctgtcgacgatgtttttactgagcttaatttaccaagaatcaacaaatggcagtcccaaggtggtcattgcggtgttggtgatgctaattacgtaccagaacccaatctgtggactcaggaccagctcagcttgacaaaccaagacttgcactccaatgtgcacaacccagtgattgagcagatcgaaacctcatcaggagtcagattgtag

SEQ ID NO: 12 - DNA, 1026 bp, Pichia pastoris
atggtgcataaggctgaatacttggacgaccacccaactcagatttccagcattctttcaggaggttacaaccacccattacttcgtgaatggcaacatgaacgtcaactcaacaaaaacatgttcatctttcccctgtttgtcacagatcgaccagacgaagaagaacttattcctagtctacctaatatcaagaggtttggcgttaacaagttgattccttatgtaggaggtttggtttccaaaggattgagggcggtgatcctatttggtgttcctctgaagcccggtgtgaaagatgaagaaggaacggccgctgatgatccagagggacctgttatccaagccatcaaacacttgagaaagaactttcctgacctgtatatcatcaccgatgtctgtctatgtgagtacaccagccatggacattgtggaatactatatgaggatggcactatcaacagagagctctcagtccgtcgtattgctgctgtagctgtcaaatatgctcaagctggagccaactctgtggctccttctgatatgactgacggcagaataagagatattaaagaaggcttactaagtgcaggactggcacataaaacgtttgttatgtcctacgctgcaaaattctctggtaatttgtatggccctttcagagatgctgcaggttcctgtccatctcaaggggacagaaaatgttaccagcttccttctggaggaaaagggttggcccatcgtgctctgattcgtgatatgaatgaaggcactgatggaattattgtcaaaccatctacattctatttggacattgtcgctgatgcttatcagctttgtaaagactatcctatctgctgttaccaggtttctggagagtacgccatgctacatgcagcggcagagaagaatattgttgatctgaaatcaatcgcttttgaagctcatcaaggattcttgcgggctggagctcgtttaatcattagttactttacccctgaattcctggagtggttatctgaatga

SEQ ID NO: 13 - DNA, 1035 bp, Pichia pastoris
atgaaccaaatcgaacagagcggacccattgattgcagttccttgaaattggggtcccgaaagtccgctctggctataatccaggcagaaatcgtccgccaattgatattgaaagaataccctgaattggagacgaagttggtcagtgtgtccaccctgggggaccaagtccagaataaagcacttttcacgtttggaggaaaatctttgtggaccaaagaacttgagatgttgttgttggagagtgtgggaggatttgaccaaatagacatgattgtacactcgttgaaagacatgccaactcatttaccagacgaatttgagctgggttgcattattgaaagagaagaccctagagacgctttggtcgtgcaagatggtttatcttacaagtcattggccgaccttccagagggagctgtggtcggtacgtcttcggttagaagatcggctcaactactgaagaatttccctcatctgaaattcaaatctgttagaggaaaccttcagaccagactaagaaaattagatgatccagattccgagtactgctgtctcctccttgcagcagccggtttaatcaggacaggcttacaacacagaatttcaatgtatttgaacgacgatgtgatgtaccactccgtcggacaaggagcattaggagtagagatcagaaaaggtgaccaattcatgaaaaatatctgtgaaaagattgggcatagaaccaccacccttcgttgtcttgcagagagagcactgctgagatatctagagggaggctgctcggtgccaattggggtctccactatttatagcgaggatacgaaggaacttaccatgaactccctagtcgtcagttgtaacggtcgtgactcggtaacagaatcaatgactgaagtcgtgactactgaagagcaagctgaagatttcggtgaaaggctggcccagaagctcatagatcaaggtgcgaaacgcattcttgacgagatcaacttcaacaagatcaaagagattaaggaagagggtttacattaa

SEQ ID NO: 14 - DNA, 798 bp, Pichia pastoris
atgccaaaagccattcttctgaagaataaaactacaccgaaggatccttatctggagaacttcgtaagtagtggctactcgaccgatttcgtaccacttttagatcatattcacatggagaaatctgagatcatcgcatttctcaagactgactactttttgcataaaactttggcgtttattattacgtcccaaagagctgtagaaatgctgaatgagtgtatgcaaatactgagacgtactgatcctgaaattacacaaatcatctatagtaaacctgtctatacagttggccctgccacctacagaatacttgcggatgctggcttcgtggatctacgaggcggagataaggcaggaaacggatccattctagcccagataattttgaatgatgacatttacactggaattgaagattctgacaagcatataacgtttttcacgggagaaacaaggagagacataattcccaaatgtttactctctaacaactttcaactttacgaaaagattgtctacaagactcttcctagggatgatatcgtgactagattcaagtctgccgttgacagcatcgaccaatcgcaaagaagttccagttgggtggtcttcttttcgcctcaaggaacagaggacattgtaacgtatcttcaacacaccaaagaccaatttaatattgcatctatcgggccaaccacagaaaaataccttctaagcaaaaacctgaaaccaaaagttgtggcacctaagccagagcctatctctttactattgtctatacaaaaagtgcactaa

SEQ ID NO: 15 - DNA, 1086 bp, Pichia pastoris
atgagtagatttccagaactgaagaatgaccttattttaagggcagctcgtggtgaaaaagttgaacgtcccccaatatggattatgagacaggccggaagatatcttccggagtaccatgaggtcaaaggaggtagggacttctttgaaacttgcagggatgctgagattgcttctgaaattactatccagccgattacgcattttgacggtctgatcgatgcagctattatcttcagtgatatcttggtgattcctcaagctatgggcatggaagttaagatggtggacaaagttggcccacagttccccaatccgctaagaaaaccgtctgacttggatcatttgaaaaaagacgttgacgttttgaaggaactcgattgggccttcaaagctatctcattgaccagaaaaaaactcaatggacgagtgcctttgcttggattttgtggtgctccttggactctactggtttatatgactgaaggaggcggtaccaagatgtttcgatttgcaaaagagtggatctacaagtttaccaaggaatctcatcaattactccaacagatcactgacgttgcagttgaattcttagctcagcaagttgttgcaggtgcccaaatgttacaagtttttgaatcttggggcggtgaattggggcctgatgaattcgatgagttttctttgccttatttgagacagatttcctctaaacttcccctgaggttgaaggaacttggaatcacagagaatgttcccataactgtctttgctaaaggctcttggtacgccttggagcaattgtgcgacagtggttatgatgttgtctcgttggattggttattccgtccaagtgatgctgtccagattgctaacggaagaatcgcattgcaaggtaatcttgaccctggaaccatgtacggctccaaagaaaccatttccaagaaagtggacaaaatgatcaagggttttggtggaggaaagcaaaactacataattaattttggacacggcactcatccattcatggatccagaacagatcagatggttcttacaagaatgtcatcgcattggatctcaatag

SEQ ID NO: 16 - DNA, 978 bp, Pichia pastoris
atggccatcgactctgatatcaatctaagctctcccaatgattccatccgtcaaaggatgttcgagcttatccagcggaagcaactcgaaattgtcgctgcattggaggcaattgaaggaaacgataccaaatttcgttctgattcttgggaaagaggagccgaaggtggaggaggaagatctatgcttattcaagatggaagagtgtttgaaaaggctggtgtaaatatttccaaggttcatggcgtattgcctcctcaagctgtgagccagatgagaaatgaccactccaagctagatctgcctgcgggaacctctctgaagttctttgcctgtgggctttcgttggtcattcatccccataatccccatgctccaactacccatctgaattatcgctacttcgaaacttgggatgaaactggaaagcctcacacctggtggtttgggggcggtgctgatttaacgccttcgtacctgtatcccgaggatgccaagcaattccatcaagcccataaggatgccctggacaaacacgatgttagcttgtacccgagattcaaaaagtggtgtgatgaatactttctgatcaaacatcgaaatgaaactagaggtattgggggtattttctttgatgattttgacgagtttgatgctgagaggtccctgaagttggttgaagattgtttcaatgctttcttggaatcttatcccgctatcactcgaaaaaggatggacaccccttcaactgatgctgagaagaactggcaacaaattagaagaggaagatatgtcgaattcaacttagtattggatagaggtactcaatttggtttgagaacgcctggatctcgtgttgaaagtattttgatgtcgttgccaagaacagctggttgggtctatgatcatcatccagagcctggctccagagaagaggagttattgcaggtactacaaaatcctattgaatgggtatga

SEQ ID NO: 17 - DNA, 1683 bp, Pichia pastoris
atgctgaaaagtcttgcaccaaattcctcaattgccgttttaggttcagggatatctggattgactttcagcttttttttgaatcggttgcgtcccgatgttaagatccatatctttgaaaaatccaagcaggttggaggatggatcagatcagaagagcatgaaacttttcattttgaaaagggacccagaactttgagaggcacaaatacgggtaccttgatgttgttggatcttcttaccaagataggagcaaatgacaaggtcctgggactgcacaaagattctcttgctaataaaaagtatctgttgtccccgttctcagatgttcacggaaacaacgcaaagcttcttcaagtgccacaggatttcagctcttttgtaaagttcatgtttgacccgttgtctaaggatctcattctcggtcttttgaaagaaccatggcaaccaaaattaaagtattcagatgagtcggttgaccattttttcaacagaagatttgctaccaaactatcagagaatatcgtcagcgcaattgtgcatggaatctatgcgggcgacgtgaagaagttaagtgtgaaagccatcttccctaggctccctgagatggaacaggaaagtggctctattataaggtatatgatcgcccaatacaggacaaaaaagaacgtcaaacaaaaagttgacccttttttggcagattatgaaaaattgatcggtacatctttgagtttcaaaaatatttctttgtttctgaaaaactttcccatgctgagttttcagggtggactacagaaacttcccatctcattgaagaaccatttatcacagattgaaaacatcaagtttcattttgacagcaaaatcaaaaacattgctttggagagcggtaaggtggcattgactgaccatgatcaggtttatcttgttgaccatgtgagatctaccattaataccaacgaattggccaaaatcatttcacccgttgttccaagttctactaagaaaaaatccgttttcaaatccaaagcgaatggcccagggctggtcaaatgtttgagctggctacactatacaaatatactaatgtgcaacatttatatacctaagcacgtctcaaaatctatcaccggatttggatacttggttcctcgatcaatgtcttctcaggcatccaaacttctcggtgtcatatttgactcagacatcgagactgcaatgactcctaattttacagaggccaacattacggcgataaacagtaactctgcatctcccaagcaactccaaaagttttctgaccaattcgtcaataatgatctccctaaatacaccaagttgacgctaatgcttggaggtcattatctcaagtcggaggcagacatgcccggttccgcagagagtaaacatgctgtcaaggcgattctgtcaaatcacctgaatattgatctagatgagtttgcatctttgccagacttcaagatggaaatcaccaagatccccaactgcattccccaatatgaagttgggtatcttgatctcaagagaaaggttcagaatgcagcctccaaagagttcaacgaccaaataagttttggaggcatggcatttggtgatggtgtggggatccctgactgtgtccagaatgcattcaaagattcggctaccctcagtggcatttaa

SEQ ID NO: 18 - DNA, 1125 bp, Pichia pastoris
atgcttaaccgtcgtttccaatctaccgtgtcctcgagtctgaacaagggcactggaatagtgttcatgaatatgggtggtccctccactgtcaaggaaacctatgactttttatttcgtcttttctcggacggagatttaatcccgtttggcagatttcagaacatcctggcccgcttcattgcaagtagaagaacacccaaaattgaatcctactacaaagctatcggaggtgggtctcctatccgaaagtggtctgaataccagagttctaaactatgtgaaaaattagacattatcagtccacaatcggctcctcataagccttatgttgccttcagatacgctaatcctctcactgaagatactttacaaaagatgaaaaatgatggaattactaaggccattgccttttctcaatatccgcaatttagttattcaaccaccggatcatcgattaacgaactttacaggcaatcgaaaattttggaccctgatcaatctattaaatggacagttatagatcgctggcctgaccacccagccttagttaaaactttcgcagctcatatcaaagatactctaaacagattcaaaactgaaaatggactgactgacacaaaagacgtcgtcctccaattcagtgctcattctttaccaatggatattgtcaataaaggagattcgtatcctgcagaagtcgcagcgagtgtctttgccattatgaaagaacttaacttctcaaatccttataaattaacctggcaatcacaggttggcccaaagccttggctgggtgctcaaactgaaaaaattaccaagcagctagcatccagtgatgttcctggagtcgttttggttcctattgcctttacctctgatcatattgaaactctccatgaactggatattgaactgattcaagaactacctaatccttcaaaagtaaagcgagttgaatcgttgaacggagaccaaactttcattgactccttggcagaactagtgaagagtcacattgattcgaaggttgtattttccaaccagttgccattggattccatgctgggagtagtgtcagataattccctcacagatccaaaagagtttttcagagcccattga

SEQ ID NO: 19 - DNA, 30 bp, Artificial Sequence
  Synthetic oligonucleotide
gagggtctcggatggagtttgtcgcccgtc

SEQ ID NO: 20 - DNA, 34 bp, Artificial Sequence
  Synthetic oligonucleotide
gagggtctcgattacaatctgactcctgatgagg

SEQ ID NO: 21 - DNA, 35 bp, Artificial Sequence
  Synthetic oligonucleotide
gagggtctcggatggtgcataaggctgaatacttg

SEQ ID NO: 22 - DNA, 33 bp, Artificial Sequence
  Synthetic oligonucleotide
gagggtctcgattattcagataaccactccagg

SEQ ID NO: 23 - DNA, 35 bp, Artificial Sequence
  Synthetic oligonucleotide
gagggtctcggatgccaaaagccattcttctgaag

SEQ ID NO: 24 - DNA, 33 bp, Artificial Sequence
  Synthetic oligonucleotide
gagggtctcgattagtgcactttttgtatagac

SEQ ID NO: 25 - DNA, 35 bp, Artificial Sequence
  Synthetic oligonucleotide
gagggtctcggatgagtagatttccagaactgaag

SEQ ID NO: 26 - DNA, 29 bp, Artificial Sequence
  Synthetic oligonucleotide
gagggtctcgattattgagatccaatgcg

SEQ ID NO: 27 - DNA, 32 bp, Artificial Sequence
  Synthetic oligonucleotide
gagggtctcggatggccatcgactctgatatc

SEQ ID NO: 28 - DNA, 31 bp, Artificial Sequence
  Synthetic oligonucleotide
gagggtctcgattatacccattcaataggat

SEQ ID NO: 29 - DNA, 34 bp, Artificial Sequence
  Synthetic oligonucleotide
gagggtctcggatgctgaaaagtcttgcaccaaa

SEQ ID NO: 30 - DNA, 32 bp, Artificial Sequence
  Synthetic oligonucleotide
gagggtctcgattaaatgccactgagggtagc

SEQ ID NO: 31 - DNA, 34 bp, Artificial Sequence
  Synthetic oligonucleotide
caatcgctagcatccaacatccaaagacgaaagg

SEQ ID NO: 32 - DNA, 42 bp, Artificial Sequence
  Synthetic oligonucleotide
ggatagcatgcaccttatcaagatagctagaaatagaaatgg

SEQ ID NO: 33 - DNA, 37 bp, Artificial Sequence
  Synthetic oligonucleotide
caatagcatgcaacatccaaagacgaaaggttgaatg

SEQ ID NO: 34 - DNA, 43 bp, Artificial Sequence
  Synthetic oligonucleotide
catggtaccggtaccttatcaagatagctagaaatagaaatgg

SEQ ID NO: 35 - DNA, 34 bp, Artificial Sequence; identical to SEQ ID NO: 31
  Synthetic oligonucleotide

SEQ ID NO: 36 - DNA, 43 bp, Artificial Sequence
  Synthetic oligonucleotide
gatattgctcgagaccttatcaagatagctagaaatagaaatg

SEQ ID NO: 37 - DNA, 32 bp, Artificial Sequence
  Synthetic oligonucleotide
caatctcgagaacatccaaagacgaaaggttg

SEQ ID NO: 38 - DNA, 44 bp, Artificial Sequence
  Synthetic oligonucleotide
caaccatttctatttctagctatcttgataaggtcttaagtcca

SEQ ID NO: 39 - DNA, 43 bp, Artificial Sequence; identical to SEQ ID NO: 34
  Synthetic oligonucleotide

SEQ ID NO: 40 - DNA, 34 bp, Artificial Sequence
  Synthetic oligonucleotide
ttacttaagtccaacatccaaagacgaaaggttg

SEQ ID NO: 41 - DNA, 22 bp, Artificial Sequence
  Synthetic oligonucleotide
tcacagacgcgttgaattgtcc

SEQ ID NO: 42 - DNA, 39 bp, Artificial Sequence
  Synthetic oligonucleotide
ttgctcctcagcttagaagaactcgtccaacatcaagtg

SEQ ID NO: 43 - DNA, 24 bp, Artificial Sequence
  Synthetic oligonucleotide
ttagtcttgctcctcagcttagcc

SEQ ID NO: 44 - DNA, 22 bp, Artificial Sequence
  Synthetic oligonucleotide
tcacagacgcgttgaattgtcc

SEQ ID NO: 45 - DNA, 37 bp, Artificial Sequence
  Synthetic oligonucleotide
ttttgcggccgcatgagcaatctacccccaacttttg

SEQ ID NO: 46 - DNA, 36 bp, Artificial Sequence
  Synthetic oligonucleotide
aaaagcggccgcctagacaccaccatctagtcggtt

SEQ ID NO: 47 - DNA, 45 bp, Artificial Sequence
  Synthetic oligonucleotide
actagatggtggtgtctagtcaagaggatgtcagaatgccatttg

SEQ ID NO: 48 - DNA, 46 bp, Artificial Sequence
  Synthetic oligonucleotide
tctgacatcctcttgactagacaccaccatctagtcggttttctag

SEQ ID NO: 49 - DNA, 27 bp, Artificial Sequence
  Synthetic oligonucleotide
aaacgctgtcttggaacctaatatgac

SEQ ID NO: 50 - DNA, 24 bp, Artificial Sequence
  Synthetic oligonucleotide
aaactgtcagttttgggccatttg

SEQ ID NO: 51 - DNA, 25 bp, Artificial Sequence
  Synthetic oligonucleotide
acgctgtcttggaacctaatatgac

SEQ ID NO: 52 - DNA, 31 bp, Artificial Sequence
  Synthetic oligonucleotide
tacccattcaataggattttgtagtacctgc

SEQ ID NO: 53 - DNA, 20 bp, Artificial Sequence
  Synthetic oligonucleotide
gagcttcttctacggccccc

SEQ ID NO: 54 - DNA, 27 bp, Artificial Sequence
  Synthetic oligonucleotide
tccagcagagtaaaatttcctagggac

SEQ ID NO: 55 - DNA, 34 bp, Artificial Sequence
  Synthetic oligonucleotide
ctcttttaggttttaagttgtgggaacagtaaca

SEQ ID NO: 56 - DNA, 20 bp, Artificial Sequence
  Synthetic oligonucleotide
gtgggtgcttctttgcgtgg

SEQ ID NO: 57 - DNA, 27 bp, Artificial Sequence
  Synthetic oligonucleotide
agaattgccatcaagagactcaggact

SEQ ID NO: 58 - DNA, 32 bp, Artificial Sequence
  Synthetic oligonucleotide
gatagagagaaatcgcaaactttgagaggaag